European Patent Application EP 4 660 309 A1, published December 10, 2025. Title: TRANSFORMED MICROORGANISM AND POLYHYDROXYALKANOATE COPOLYMER PRODUCTION METHOD. Applicant: KANEKA CORPORATION. Application JP. The sequence listing filed with the application follows.

SEQUENCE LISTING (45 sequences)

SEQ ID NO: 1 - protein, 562 aa, Mycobacterium cookii
MTTTAKVDELAAPLDLLLTSATKPFASRMMPNATWARFAGNLAQHPGAVADRVGALTRELGNIAVGKSHRAPGRADKRFSDPAWQENPLLHRIMQAYLAGSETAEELLADAQLDWRDKEKMQFVIDNFVEGLAPSNNPLISPLGWKALIDTGGLSAVRGARAFARDMLSKPRVPAMIEPDAYAVGEDLAVTKGAVVLQTSVFELIQYAPQTPKVRAIPLLMVPPVINKYYVMDIAPGRSMIEYFVQQGQQVFTISWRNPQARHRDWGFDTYGAAIVEAMDAAEKITGTDSTHLLATCSGGILAAMTAAHLAEIGEGDRVAGLNLAVTVLDETRAGFAAAAMSDRAAQAAIRVSSRKGFLDGRDMAEMFAWLRPTDLVWRYVVNNYVQGRKPAAFDVLFWNADTTRMAAALHRDLVLMGLRNALVTPGGVSMLGSPVDLGKITADAYIVGGIADHISPWQATYRSARLLGSKDNRYVLSTNGHIAALVNPPGNPKASFRTGSVDAEDAQQWLDSAEKHADSWWPDYTAWLAERSGAEVDAPKALGGEDLPPLGPAPGSYVMEK

SEQ ID NO: 2 - protein, 566 aa, Mycobacterium persicum
MRPEITDRSGQVQNVGLDQLLTEAASAESRFVPGAEFLKAAGGLALRPRLLANQTATVAADLARVIAGRSGRTPPKGDSRFRDPAWTQSWLFRRICQGYLSISDYARALADESGLDWADHERLRLVVDNLIDALAPTNFPLTNPTVWKTTIDRGGENFVTGARAAVRDARSPIKLPASVDRTPFEVGKTMAASPGAVVRRDDRFELIQYEPRAEEVHKVPVLLIPPMISKFYVVDLSPGKSMVEFLGDRGLQPFALSWANPTRDNAGWNLQDYLESIVEAIETTREIAGADAVHVVAFCAGGIATTTAVAHLAALGHIDRVASLSLMVTVLDVRRGGPILSIASPDVAKAAKAKIKRKGYLAGTELSRTFAWLRPNDMVWNNFVNNYYLGNKPPALDLLFWNLDSMNMPAGLHADLVDLALANPLANPGALRVLGTPIDLAQITCDAYIAAGETDHLTPWPSCYRSVEMLGGKTRFALSTSGHIAAVIHPPGNPKSAYRIGDESCPTPEEWLRSAQVHKGTWWQDWAPWLAERAGEKTTAPDRLGNSRYTPLDPAPGTYVFKQSQG

SEQ ID NO: 3 - protein, 562 aa, Mycolicibacterium insubricum
MTGENTAAEEVAAPLDMLLIRSATGFGRRMVPNGAWVRTAGNLIKRPGTVASRVGALVGELTDIALGASDRAPGRADKRFADPAWSQNPVLQRVMQTYLATSETAQHLLDDAELDWRDREQMQFVIDNVVEGGSPSNNILLSPLGWKAMIDTGGLSAVRGARNFVRDMRSAPRVPAMVDANAFAVGDSLAVTPGSVVLKTRVFELIQYAPATPTVTTVPLLVIPPVINKYYVLDLAPHRSLMEYLVSQGIQPFVLSWRNPHKRHRDWGFDTYGGSMIEAMDAIGDITGSDRVHLLGTCSGGMLASMVAAHLTAIGQGERLASLALAVTVLDQSKAGFAAAALDEKSGQAAIRKSARKGYLDGAALAEVFAWLRPTDLVWRYWVNNYIQGRDPAAFDVLYWNADTTRMTAALHRDMVTTGMTNALAHPGAATMLGTEVDLSKVTADIYVVGGVTDHICPWPATYRSSRLFGSDDVRYVLSSSGHIAAIVNPPGNPRASFRFGPPDSESHEEWAESAEKAADSWWPDYAAWLKQRGEDKDAPDSLGSKAFPVRSPAPGEYVHEH

SEQ ID NO: 4 - protein, 572 aa, Nocardioides sp.
MTTTEEEAAAAAEGSSLAEELSTPLDLLLADAGRSPIRRFLPGMSGVRFAAGLARRPHKVVGRTAGLGVELAKVGLGRSELAPAPKDRRWADEAWAKNPLFRRTLQGYLAWGQAVRGLVDDADLDWGDGHRIGFLADNLVEAMAPTNNPALNPKVLKRTLDTGGGNLLEGGKRLVRDFATAPRVPSMVEADAFEVGKDIAVTPGAVVLRTDVFELIQYSPQTPQVREVPLLIVPPTINKYYVVDLAAERSMIEHLVRSGLQVYCISWRNPDARHAAWDLDTYGQAVLDALDGIEQISRQDKTALLGICSGGMIASMVMGHLAATGKLDRVAAFSLMVTVLDQERAGVTSALLSHKAAAASTRASAEKGYLDGRVLAEVFAWLRPNDLIWNYWVNNYLMGHAPKAFDILFWNADPVRMSAGMHRDFMDLAFRNALVEPNAATMLDTPVDLGKVTTDSYVVAGIADHLCQWESCYASTQLLGGTSKFVLSTSGHIAAMVNPPGNPKANFRTAEQNPPEAQDWLAGAHQVPGSWWDDYAGWLAERCGDERGKPRRLGSAQHEPLCEAPGTYVHDR

SEQ ID NO: 5 - protein, 151 aa, Pseudomonas putida
MPHVPVTELSQYVGKELGHSEWLKIDQQRINLFAEATGDFQFIHVDPEKAAKTPFGGTIAHGFLTLSLIPKLIEDILVLPQGLKMVVNYGLDSVRFIQPVKVDSRVRLKVKLGEVVEKKPGQWLLKAIATLEIEGEEKPAYIAESLSLCFV

SEQ ID NO: 6 - protein, 151 aa, Pseudomonas aeruginosa
MPFVPVAALKDYVGKDLGHSEWLTIDQERVDQFAECTGDHQFIHVDPEKAAKTPFGGTIAHGFLSLSLIPKLMEGLLVLPEGLKMAVNYGLDTVRFIQPVRVGSRVRLGLTLLDVNEKNPGQWLIKARATLEIEGQEKPAYIAETLSLCFV

SEQ ID NO: 7 - protein, 598 aa, Drosophila melanogaster
MSSSDGKLRYDGRVAVVTGAGAGLGREYALLFAERGAKVVVNDLGGTHSGDGASQRAADIVVDEIRKAGGEAVADYNSVIDGAKVIETAIKAFGRVDILVNNAGILRDRSLVKTSEQDWNLVNDVHLKGSFKCTQAAFPYMKKQNYGRIIMTSSNSGIYGNFGQVNYTAAKMGLIGLANTVAIEGARNNVLCNVIVPTAASRMTEGILPDILFNELKPKLIAPVVAYLCHESCEDNGSYIESAAGWATKLHMVRGKGAVLRPSLDDPVTIEYVKDVWSNVTDMSKAKHLGAIAEASGTLLEVLEKLKEGGGDAIEDAFEFNSKELITYALGIGASVKNAKDMRFLYENDADFAAIPTFFVLPGLLLQMSTDKLLSKALPNSQVDFSNILHGEQYLEIVDDLPTSGTLLTNGKVFDVMDKGSGAVVVTNSESFDESGRLLVRNQSTTFIVGAGKFGGKKDPIAGVVPLQPAPNRQPDATVQYTTSEDQAALYRLSGDKNPLHIDPQMALLAGFKTPILHGLCTLGFSVRAVLAQFADNNPALFKAVKVRFSGPVIPGQTLRVDLWKQGTRINFRTVVVETGKEVISGAYVDLKSSQAKL

SEQ ID NO: 8 - protein, 394 aa, Cupriavidus necator
MTREVVVVSGVRTAIGTFGGSLKDVAPAELGALVVREALARAQVSGDDVGHVVFGNVIQTEPRDMYLGRVAAVNGGVTINAPALTVNRLCGSGLQAIVSAAQTILLGDTDVAIGGGAESMSRAPYLAPAARWGARMGDAGLVDMMLGALHDPFHRIHMGVTAENVAKEYDISRAQQDEAALESHRRASAAIKAGYFKDQIVPVVSKGRKGDVTFDTDEHVRHDATIDDMTKLRPVFVKENGTVTAGNASGLNDAAAAVVMMERAEAERRGLKPLARLVSYGHAGVDPKAMGIGPVPATKIALERAGLQVSDLDVIEANEAFAAQACAVTKALGLDPAKVNPNGSGISLGHPIGATGALITVKALHELNRVQGRYALVTMCIGGGQGIAAIFERI

SEQ ID NO: 9 - protein, 392 aa, Cupriavidus necator
MNEAVIVSTARTPLAKSWKGAFNMTHGATLGGHAVQHAIARAKIEAAEVEDVLMGCANPEGATGANIARQIALRAGCPVTVPGATVNRFCSSGLQTIAMAAQRVIADEGDIFVAGGVESISCVQQEMNRHMVQESWLLKNKPEIYWNMLQTAENVAKRYNISKERQDEYGVRSQQRAAAGQEAGKFKDEIVPMTVLAGVADKSTGQLVTKEVTVSADEGIRADTTLEGVSKIRSAVPGGVITAGNASQFSDGASAAVVMNARVAEARGLQPLGVFRGFAVAGCEPDEMGIGPVFAVPKLLKKAGLKVDDIGLWELNEAFAVQVLYCADTLGIPMDRLNVNGGAIAVGHPYGVSGARLVGHALIEGKRRGVKYVVVTMCIGGGQGAAGLFEVL

SEQ ID NO: 10 - DNA, 1056 bp, synthetic construct
  source 1..1056: mol_type = other DNA
gcgcgcatttaaatctgccaccacgttgtgctcggtgatcgccatcatcagcgccacgtagagccagccaatggccacgatgtacatcaaaaattcatccttctcgcctatgctctggggcctcggcagatgcgagcgctgcataccgtccggtaggtcgggaagcgtgcagtgccgaggcggattcccgcattgacagcgcgtgcgttgcaaggcaacaatggactcaaatgtctcggaatcgctgacgattcccaggtttctccggcaagcatagcgcatggcgtctccatgcgagaatgtcgcgcttgccggataaaaggggagccgctatcggaatggacgcaagccacggccgcagcaggtgcggtcgagggcttccagccagttccagggcagatgtgccggcagaccctcccgctttgggggaggcgcaagccgggtccattcggatagcatctccccatgcaaagtgccggccagggcaatgcccggagccggttcgaatagtgacggcagagagacaatcaaatccgcttgcatgagtgccggcgtgcgtcatgcacggcgccggcaggcctgcaggttccctcccgtttccattgaaaggactacacaatgactgacgttgtcatcgtatccgccgcccgcaccgcggtcggcaagtttggcggctcgctggccaagatcccggcaccggaactgggtgccgtggtcatcaaggccgcgctggagcgcgccggcgtcaagccggagcaggtgagcgaagtcatcatgggccaggtgctgaccgccggttcgggccagaaccccgcacgccaggccgcgatcaaggccggcctgccggcgatggtgccggccatgaccatcaacaaggtgtgcggctcgggcctgaaggccgtgatgctggccgccaacgcgatcatggcgggcgacgccgagatcgtggtggccggcggccaggaaaacatgagcgccgccccgcacgtgctgccgggctcgcgcgatggtttccgcatgggcgatgccaagctggtcgacaatttaaatgcgcgc

SEQ ID NO: 11 - DNA, 869 bp, synthetic construct
  source 1..869: mol_type = other DNA
gcgcgcatttaaatcgaggaagagatcctggcctttgcccgccagtacgatccgcagccgttccatatcgacaaggaagccgctgccaggagcatctatggcggcgtgatctcgagcggctggatgacgtgctcgatcatgatgcggctgctggtgctgagcaccaccggcaagtcggccagcatgggctcgcctggcgtggacgagatccgctggctcaagcccgtctacgccggcgacacgctcaccgtcgtgctgaatgtgctcgatacccggccgtcgcagtccaagccggaccgcggcgtggtccacacccagtgggaagccaccaaccagcgcggcgaactggtctgcaccgtcaagggcatgggcatgtacggccgccgccccgcttaagaacactttatcgtcaagaggagactatcgaccggatacgcagttttgacgcggtgcgacaatatgccacacaggcatgtcgcgcccctggaggccgcctgatgcgcggctttctgcatttttaggaaccgatttgtgacgttgatgcctgtcaaatgctgcttcgcggatttgtgcgtcgattgtccgttctgctgaacagtgtgttctgtgccgttgggtttacccctaatgttgcgttgcggtacagtcgcgcccacgatgttttatgtgttgcgctccccggccgaaaaccgcgcttgccatgaaggcaagtccgtcgggaagtgcaaaaacctcgtattccaacgctacccggccgccgtactgagccgggaccgttcgcggtttcggccaggtgccgcagcgccggcaaggtcctacagggcctgcagcgcacgcagtcagttgtccttccgtatttaaatgcgcgc

SEQ ID NO: 12 - DNA, 1009 bp, synthetic construct
  source 1..1009: mol_type = other DNA
gcgcgcatttaaatggagttccagaccctgctcgactttatcgccgaagccgaactggaccgcgtcggctgcttcgcctactcgccggtggagggcgccaccgccaatgacctgccgggcgcgctgcccgacgaggtgcgcgaggaacgccgcgcccgcttcatggaagtggccgaagaggtctcggcgcgccgcctgcagcgcaaggtcggccagaccctgcgcgtgctggtggacgaggtcaaccaggatggcggcatcggccgttcgtccgcggatgcgccggaaatcgacggcctcgtctatatcgcgccgccggaacgccacgcccagcgctatcgcgccggcgagttcgtcgacgtgaagatcaccggcgccgatggccacgacctgtggggcgcggtctgaaacgggttgattaggtaaaagtacgctcgttcgatttcgtccgcgtcccgctatactgtgcggtgcaacataacctcatggagacaaagtcggttagccttgcgccttgcttcgctgacgaagaacctctgcgcgctcggcctggccgccgtgctcgcgctggcgggcacggcgcaggcagcgccggcgaccgagctgtcgaccggcccggttaacaccgggccagccggcggcgaaggcctgggcatcaaccaggccattcgcgacggcgaagcccggcgcggcggcacctcgctttccactggcgcgccaaaacccctggcgccgcggccggaatatgcgtcgctgccggtctacgtcggcaaggtcggcgaccagccggtgcggctgcgcctgggccccaagcctgacgagcgcgacagcgtgcgtggcgaatacgccggccgtggcgccggtgtgcgcctgctggcaggcgagtgggaggacggcgccttcctgatggaggagtccgacgacggcacccgcgtatcgggcaactgggaaggcagcatcgacgccagcggcgccgtgcgcggcacctggaccgaatttaaatgcgcgc

SEQ ID NO: 13 - DNA, 825 bp, synthetic construct
  source 1..825: mol_type = other DNA
atccatttaaattgcatgcgggcttgcacgtgccgcatgcgcggctggtgatccgcaagggccaccatgccgacgtggacagctactccgccttcctggaggcggaccgcaccacgcgcaccgggctggccggctacctgcgcgagcatggcgtcaggcgcgtgttctgcgcgggtctggcgacggactactgcgtggcctggagcgcgctcgatgcacgcgccgcgggcttcgcggccgcggtgatcgaggatgcctgccgcgccatcgacctggaagggtcgctggccaaagcatggcaggacctcggcgccgccggcgttgcgcgcgtcacgtccgctgaactgctcaagggccagggctgaaccgaaccaccgaactgaacgacacaagagaatccgaggagcaagacatgtcggctgcgggcaccgcgcgggccacgcccgccgacatgctcgcctggggccgggaggtgctggccagccagcccttctcggtcctggtcggcaccgaactggcggcgttgtcgccgggcaaggctgagttgcgcctgccgatccgtcaggacctgcggcagcagcacggcttcctgcacggcggcgtggtcagctacctggccgacaatgcgctgacctacgcgggcggcgcggccatggcggtgccggtcgtgacatccgagtacaagatcaactacgtgcgcccggcgatcggcgagctgctggtcgcccgcgccgaatgcgtcagcgccggccgccagcaggcggtggtgcgctgcgacgtgtacgtcgtcagggatggcgaggagaggctctgatttaaatccga

SEQ ID NO: 14 - DNA, 29 bp, synthetic construct
  source 1..29: mol_type = other DNA
ttgacaattaatcatccggctcgtataat

SEQ ID NO: 15 - DNA, 1579 bp, synthetic construct
  source 1..1579: mol_type = other DNA
gcgcgcatttaaatcgaggaagagatcctggcctttgcccgccagtacgatccgcagccgttccatatcgacaaggaagccgctgccaggagcatctatggcggcgtgatctcgagcggctggatgacgtgctcgatcatgatgcggctgctggtgctgagcaccaccggcaagtcggccagcatgggctcgcctggcgtggacgagatccgctggctcaagcccgtctacgccggcgacacgctcaccgtcgtgctgaatgtgctcgatacccggccgtcgcagtccaagccggaccgcggcgtggtccacacccagtgggaagccaccaaccagcgcggcgaactggtctgcaccgtcaagggcatgggcatgtacggccgccgccccgcttaagaacactttatcgtcaagaggagactatcgactgcttctggcgtcaggcagccatcggaagctgtggtatggctgtgcaggtcgtaaatcactgcataattcgtgtcgctcaaggcgcactcccgttctggataatgttttttgcgccgacatcataacggttctggcaaatattctgaaatgagctgttgacaattaatcatccggctcgtataatgtgtggaattgtgagcggataacaatttcacacaggaaacaattgcacgtgcagagagacaatcaaatcatgccccatgtaccggttacagagctttcgcagtacgttggcaaggagctgggccactcggagtggttgaagatcgaccagcagcgcatcaacctgttcgccgaggcgaccggcgatttccagttcatccatgtcgaccctgagaaggcggcaaaaaccccgtttggcggcacgatcgcccatggtttcctgaccttgtcgctgatccccaagctgatcgaggacatcctcgtcctgccgcaaggactgaagatggtggtgaactacgggctggacagcgtgcgcttcattcagccggtcaaggtcgacagccgggttcggctgaaggtaaagctgggcgaggtggtggagaaaaagccggggcagtggctactcaaggcgattgccacgctggagattgagggtgaagagaagcctgcttatatagccgagtcgctgtcgctctgttttgtctgacggatacgcagttttgacgcggtgcgacaatatgccacacaggcatgtcgcgcccctggaggccgcctgatgcgcggctttctgcatttttaggaaccgatttgtgacgttgatgcctgtcaaatgctgcttcgcggatttgtgcgtcgattgtccgttctgctgaacagtgtgttctgtgccgttgggtttacccctaatgttgcgttgcggtacagtcgcgcccacgatgttttatgtgttgcgctccccggccgaaaaccgcgcttgccatgaaggcaagtccgtcgggaagtgcaaaaacctcgtattccaacgctacccggccgccgtactgagccgggaccgttcgcggtttcggccaggtgccgcagcgccggcaaggtcctacagggcctgcagcgcacgcagtcagttgtccttccgtatttaaatgcgcgc

SEQ ID NO: 16 - DNA, 30 bp, Escherichia coli
  source 1..30: mol_type = other DNA
tttacactttatgcttccggctcgtataat

SEQ ID NO: 17 - DNA, 1516 bp, synthetic construct
  source 1..1516: mol_type = other DNA
gcgcgcatttaaatcgaggaagagatcctggcctttgcccgccagtacgatccgcagccgttccatatcgacaaggaagccgctgccaggagcatctatggcggcgtgatctcgagcggctggatgacgtgctcgatcatgatgcggctgctggtgctgagcaccaccggcaagtcggccagcatgggctcgcctggcgtggacgagatccgctggctcaagcccgtctacgccggcgacacgctcaccgtcgtgctgaatgtgctcgatacccggccgtcgcagtccaagccggaccgcggcgtggtccacacccagtgggaagccaccaaccagcgcggcgaactggtctgcaccgtcaagggcatgggcatgtacggccgccgccccgcttaagaacactttatcgtcaagaggagactatcgaccaattggcgcaacgcaattaatgtgagttagctcactcattaggcaccccaggctttacactttatgcttccggctcgtataatgtgtggaattgtgagcggataacaatttcacacaggaaacaattgcacgtgcagagagacaatcaaatcatgccctttgtccccgtggcggcactcaaagattatgtggggaaagatctcggtcacagcgagtggctgaccattgatcaggagcgcgtggatcaatttgcggaatgcacgggcgatcatcaatttattcatgtggatcccgaaaaggccgcgaagacgccctttggtggcacgattgcgcacggttttctctccctcagcctcattcccaaactgatggaaggtctcctcgtcctgcccgaagggctcaaaatggcggtgaattatggtctcgataccgtccgttttattcaacccgtccgggtgggttcccgtgtccgtctcgggctcaccctgctcgatgtgaatgagaagaaccccggccaatggctcattaaagcccgggccacgctcgagattgaggggcaagagaaaccggcctacattgcggaaacgctctcgctctgctttgtctgacctgccggcctggttcaaccagtcggcagccgactagtcggatacgcagttttgacgcggtgcgacaatatgccacacaggcatgtcgcgcccctggaggccgcctgatgcgcggctttctgcatttttaggaaccgatttgtgacgttgatgcctgtcaaatgctgcttcgcggatttgtgcgtcgattgtccgttctgctgaacagtgtgttctgtgccgttgggtttacccctaatgttgcgttgcggtacagtcgcgcccacgatgttttatgtgttgcgctccccggccgaaaaccgcgcttgccatgaaggcaagtccgtcgggaagtgcaaaaacctcgtattccaacgctacccggccgccgtactgagccgggaccgttcgcggtttcggccaggtgccgcagcgccggcaaggtcctacagggcctgcagcgcacgcagtcagttgtccttccgtatttaaatgcgcgc

SEQ ID NO: 18 - DNA, 261 bp, synthetic construct
  source 1..261: mol_type = other DNA
tcagaaaattattttaaatttcctcttgacaggccggaataactcccatataatgcgccaccactgattgacaattaatcatcgaattagtataatagtacgcaagttcttgacactgtagcgggaaggcgttataatgcacaccccgcgcttgacagcgcgtgcgttgcaaggtataatggactcaaatgtcttgacactttatgcttccggctctataatgtgtggaattgtgagcggataacaatttcacacaggaaa

SEQ ID NO: 19 - DNA, 3001 bp, synthetic construct
  source 1..3001: mol_type = other DNA
gcgcgcatttaaatcgaggaagagatcctggcctttgcccgccagtacgatccgcagccgttccatatcgacaaggaagccgctgccaggagcatctatggcggcgtgatctcgagcggctggatgacgtgctcgatcatgatgcggctgctggtgctgagcaccaccggcaagtcggccagcatgggctcgcctggcgtggacgagatccgctggctcaagcccgtctacgccggcgacacgctcaccgtcgtgctgaatgtgctcgatacccggccgtcgcagtccaagccggaccgcggcgtggtccacacccagtgggaagccaccaaccagcgcggcgaactggtctgcaccgtcaagggcatgggcatgtacggccgccgccccgcttaagaacactttatcgtcaagaggagactatcgaccaattgtcagaaaattattttaaatttcctcttgacaggccggaataactcccatataatgcgccaccactgattgacaattaatcatcgaattagtataatagtacgcaagttcttgacactgtagcgggaaggcgttataatgcacaccccgcgcttgacagcgcgtgcgttgcaaggtataatggactcaaatgtcttgacactttatgcttccggctctataatgtgtggaattgtgagcggataacaatttcacacaggaaacaattgcacgtgcagagagacaatcaaatcatgtcctcatccgatggaaaacttcgttacgatggccgtgtggcggtggtgacgggagctggtgccggtttgggccgcgagtacgcactgctcttcgcggagcgtggcgccaaggtggtggtcaacgatctgggtggcacccactccggcgatggagcatcgcagcgggccgccgacattgtggtggatgagatccgtaaggccggcggcgaggcggtggccgactacaactcggtaatcgatggggcaaaggtcatcgagacggccatcaaagctttcggacgcgtcgatatcctggtcaacaatgccggcattctacgcgacaggagtctggtgaagaccagcgaacaggactggaatctggtcaacgatgtccatctgaagggcagctttaagtgcacccaggcggcattcccgtacatgaagaagcagaactatggccgcatcatcatgacatcgtccaactcgggcatctatggtaatttcgggcaggtcaactacactgccgccaagatgggcctcatcggattggccaacacggttgccatcgagggagcccgcaacaatgttctttgcaacgtcatcgtgccaactgccgccagtcgaatgaccgagggcattctgcccgacattctcttcaacgagctgaagcccaagctgattgctcccgtagtggcctacttgtgccacgagtcctgcgaggataatggtagctatatcgagagtgccgccggctgggccaccaagctgcacatggttcgcggcaagggcgctgtgctgcgtccttcgctggacgaccccgtgaccattgagtacgtcaaggatgtgtggtcgaatgtgaccgacatgtccaaggccaagcacttgggtgccatcgcagaggcctccggcaccctgctggaagtgcttgagaagctcaaggaaggcggcggcgacgccatcgaggatgccttcgagttcaatagcaaagagcttattacctacgccctgggcattggggcatccgtcaaaaacgcgaaggacatgcgcttcctgtacgaaaacgatgccgatttcgccgccattccaactttcttcgttctgcccggccttctgctgcaaatgtccaccgacaagctgctcagcaaggctttgcccaacagccaagtggacttcagcaacattctgcacggcgaacagtacctagagatcgttgacgatctgcccaccagtggcactttgctgaccaacggcaaggtcttcgatgttatggacaagggatccggcgccgtggtcgtcaccaatagcgagtcgttcgacgaaagtggccgcctgttggtgcgcaaccagagcaccactttcattgtcggcgctggcaaattcggaggcaagaaggatcccatcgctggtgtagttccgctgcagccggcgcccaatcgccaaccggacgcaaccgtccagtatacgaccagcgaggaccaggcggcgctgtaccgtctgtccggcgacaagaaccccctgcatatcgatccccagatggccctgctggccggcttcaagacacccatcctccatggactctgcacactgggcttctcggtgcgcgccgtgctcgctcagtttgcggacaacaacccggctctgttcaaggctgtcaaagtgcgcttctccggacccgtaattccgggccagactttgcgcgtggacttgtggaagcagggcacacgcatcaacttccgcaccgtggtcgtggagaccggcaaggaggtcatatccggcgcctatgtcgacctgaagagctcacaggccaagctgtaacctgccggcctggttcaaccagtcggcagccgactagtcggatacgcagttttgacgcggtgcgacaatatgccacacaggcatgtcgcgcccctggaggccgcctgatgcgcggctttctgcatttttaggaaccgatttgtgacgttgatgcctgtcaaatgctgcttcgcggatttgtgcgtcgattgtccgttctgctgaacagtgtgttctgtgccgttgggtttacccctaatgttgcgttgcggtacagtcgcgcccacgatgttttatgtgttgcgctccccggccgaaaaccgcgcttgccatgaaggcaagtccgtcgggaagtgcaaaaacctcgtattccaacgctacccggccgccgtactgagccgggaccgttcgcggtttcggccaggtgccgcagcgccggcaaggtcctacagggcctgcagcgcacgcagtcagttgtccttccgtatttaaatgcgcgc

SEQ ID NO: 20 - DNA, 30 bp, synthetic construct
  source 1..30: mol_type = other DNA
gggcaattggcgcaacgcaattaatgtgag

SEQ ID NO: 21 - DNA, 31 bp, synthetic construct
  source 1..31: mol_type = other DNA
gggcaattgtttcctgtgtgaaattgttatc

SEQ ID NO: 22 - protein, 559 aa, Pseudomonas sp.
MSNKNSDDLNRQASENTLGLNPVIGLRGKDLLTSARMVLTQAIKQPIHSVKHVAHFGIELKNVMFGKSKLQPESDDRRFNDPAWSQNPLYKRYLQTYLAWRKELHDWIGNSKLSEQDINRAHFVITLMTEAMAPTNSAANPAAVKRFFETGGKSLLDGLTHLAKDLVNNGGMPSQVDMGAFEVGKSLGTTEGAVVFRNDVLELIQYRPTTEQVHERPLLVVPPQINKFYVFDLSPDKSLARFCLSNNQQTFIVSWRNPTKAQREWGLSTYIDALKEAVDVVSAITGSKDINMLGACSGGITCTALLGHYAALGEKKVNALTLLVTVLDTTLDSQVALFVDEKTLEAAKRHSYQAGVLEGRDMAKVFAWMRPNDLIWNYWVNNYLLGNEPPVFDILFWNNDTTRLPAAFHGDLIEMFKNNPLVRANALEVSGTPIDLKQVTADIYSLAGTNDHITPWKSCYKSAQLFGGKVEFVLSSSGHIKSILNPPGNPKSRYMTSTDMPATANEWQENSTKHTDSWWLHWQAWQAERSGKLKKSPTSLGNKAYPSGEAAPGTYVHER

SEQ ID NO: 23 - protein, 559 aa, Pseudomonas sp.
MSNKNSDDLNRQASENTLGLNPVIGLRGKDLLTSARMVLTQAIKQPIHSVKHVAHFGIELKNVMFGKSKLQPESDDRRFNDPAWSQNPLYKRYLQTYLAWRKELHDWIGNSKLSEQDINRAHFVITLMTEAMAPTNSAANPAAVKRFFETGGKSLLDGLTHLAKDLVNNGGMPSQVDMGAFEVGKSLGTTEGAVVFRNDVLELIQYRPTTEQVHERPLLVVPPQINKFYVFDLSPDKSLARFCLSNNQQTFIVSWRNPTKAQREWGLSTYIDALKEAVDVVSAITGSKDINMLGACSGGITCTALLGHYAALGEKKVNALTLLVTVLDTTLDSQVALFVDEKTLEAAKRHSYQAGVLEGRDMAKVFAWMRPNDLIWNYWVNNYLLGNEPPVFDILFWNNDTTRLPAAFHGDLIEMFKNNPLVRANALEVSGTPIDLKQVTADIYSLAGTNDHITPWKSCYKSAQLFGGKVEFVLSSRGHIRSILNPPGNPKSRYMTSTDMPATANEWQENSTKHTDSWWLHWQAWQAERSGKLKKSPTSLGNKAYPSGEAAPGTYVHER

SEQ ID NO: 24 - protein, 559 aa, Pseudomonas sp.
MSNKNSDDLNRQASENTLGLNPVIGLRGKDLLTSARMVLTQAIKQPIHSVKHVAHFGIELKNVMFGKSKLQPESDDRRFNDPAWSQNPLYKRYLQTYLAWRKELHDWIGNSKLSEQDINRAHFVITLMTDAMAPTNSAANPAAVKRFFETGGKSLLDGLTHLAKDLVNNGGMPSQVDMGAFEVGKSLGTTEGAVVFRNDVLELIQYRPTTEQVHERPLLVVPPQINKFYVFDLSPDKSLARFCLSNNQQTFIVSWRNPTKAQREWGLSTYIDALKEAVDVVSAITGSKDINMLGACSGGITCTALLGHYAALGEKKVNALTLLVCVLDTTLDSQVALFVDEKTLEAAKRHSYQAGVLEGRDMAKVFAWMRPNDLIWNYWVNNYLLGNEPPVFDILFWNNDTTRLPAAFHGDLIEMFKNNPLVRANALEVSGTPIDLKQVTADIYSLAGTNDHITPWKSCYKSAQLFGGKVEFVLSSRGHIQSILNPPGNPKSRYMTSTDMPATANEWQENSTKHTDSWWLHWQAWQAERSGKLKKSPTSLGNKAYPSGEAAPGTYVHER

SEQ ID NO: 25 - protein, 559 aa, Pseudomonas sp.
MSNKNNDDLQRQASENTLGLNPVIGLRRKDLLTSARMVLGQAIRQPLHSAKHVAHFGLELKNVIFGKSGLQPESDDRRFNDPAWSQNPLYRRYLQTYLAWRKELHDWIDNSNLSEQDISRGHFVINLMTEAMAPTNTAANPAAVKRFFETGGKSLLDGLSNLAKDMVNNGGMPSQVNMEAFEVGKNLGTSEGAVVYRNDVLELIQYKPITEQVHSRPLLVVPPQINKFYVFDLSPEKSLARFCLRSNVQTFIVSWRNPTKTQREWGLSTYIDALKETVDVVLAITGSKDLNMLGACSGGITCTALLGHYAALGENKVNALTLLVSVLDTTLDTQVALFVDEQTLESAKRQSYQAGVLEGRDMAKVFAWMRPNDLIWNYWVNNYLLGNEPPVFDILFWNNDTTRLPAAFHGDLIELFKSNPLTRADALEVCGTPIDLKKVTADIYSLAGTTDHITPWQACYRSAQLFGGNIEFVLSNSGHIQSILNPPGNPKARYMTGSELPTQATEWQENAHKHTDSWWLHWQNWLATRSGELKKAPTRLGNRAYAAGEAAPGTYVHER

SEQ ID NO: 26 - protein, 559 aa, Pseudomonas oleovorans
MSNKNNDELQRQASENTLGLNPVIGIRRKDLLSSARTVLRQAVRQPLHSAKHVAHFGLELKNVLLGKSSLAPESDDRRFNDPAWSNNPLYRRYLQTYLAWRKELQDWIGNSDLSPQDISRGQFVINLMTEAMAPTNTLSNPAAVKRFFETGGKSLLDGLSNLAKDLVNNGGMPSQVNMDAFEVGKNLGTSEGAVVYRNDVLELIQYKPITEQVHARPLLVVPPQINKFYVFDLSPEKSLARYCLRSQQQTFIISWRNPTKAQREWGLSTYIDALKEAVDAVLAITGSKDLNMLGACSGGITCTALVGHYAALGENKVNALTLLVSVLDTTMDNQVALFVDEQTLEAAKRHSYQAGVLEGSEMAKVFAWMRPNDLIWNYWVNNYLLGNEPPVFDILFWNNDTTRLPAAFHGDLIEMFKSNPLTRPDALEVCGTPIDLKQVKCDIYSLAGTNDHITPWQSCYRSAHLFGGKIEFVLSNSGHIQSILNPPGNPKARFMTGADRPGDPVAWQENATKHADSWWLHWQSWLGERAGELEKAPTRLGNRAYAAGEASPGTYVHER

SEQ ID NO: 27 - protein, 559 aa, Pseudomonas mendocina
MSDKNNEDLKRQASENTLGLNPVIGIRGKDLLTSARMVLAQALKQPFHSAKHVAHFGLELKNVMLGQSALKPEDGDRRFADPAWSQNPLYRRYLQTYLAWRKELHDWVEHSSLSEQDASRGTFVINLMTEDMAPSNSMANPAAVKRFFETGGKSLLDGLSHLAKDMVHNGGMPSQVNMEAFEVGKNLATTDGAVVFRNDVLELIQYKPITESVHERPLLVVPPQINKFYVFDLSPDKSLARFLLRSQVQTFVVSWRNPTKAQREWGLSTYIEALKEAIDVICAITGSKDVNMLGACSGGLTTASLLGHYAALGQPKVNALTLLVSVLDTQLDTQVALFADEKTLERGQRRSYQAGVLEGSDMAKVFAWMRPNDLIWNYWVNNYLLGNEPPVFDILYWNNDTTRLPAALHGEFIEMFQTNPLTRPGALEVCGTPIDLKQVTCDFFVVAGTTDHITPWDSCYKSAHLFGGKCEFVLSNSGHIQSILNPPGNPKARYMTNSEMPLDPKAWQESSTKHADSWWLHWQSWLAERSGETKNAPRALGNKKFPAGEAAPGTYVHER

SEQ ID NO: 28 - protein, 565 aa, Rhodococcus sp.
MTKTAEPKIALVIPDATPEEEDRAGGFGARNALNAVTGVVGQGRVVLEESLRLGRELTKITVGRSDVGPAAGDRRFTDQAWTNNPIYRRVQQTYLASVDAVESVVEDLGRRVDDRHAREAAFVSTVLTSALAPTNYLPTNPAAVKEAFDTGGMSLVRGARNYVSDLRHNGGMPRMVDPDAFTVGVDLAVTPGAVVSRDEVAEVLQYTPTTETVYERPVLVVPPPIGRYYFLDLRPGRSFVEHAVSRGLQTFMLAWRNPQAEQSDWDLDTYAQRVSDAIDEVREITGSDDVNVIGFCAGGLITTALLNHLAATGDTRVHSVSYAVTMLDFADPAGLAAFSGPRLLQLVKGRSRRNGIISARDMGSAFTWMRPNDLVFNYVVNNYLMGRTPPAFDILSWNADGTNLPGALHVQFLDIFENNTLATPGAMTALGTPVDLGRITVPTFVSGAIADHLTSWKNCYRTTQLLSGDTKFVLSFSGHIASLVNPPGNPKSHYWEGGEPGPDPEAWLDAATKKTGSWWESWADWVSERAGERIVASTRLGSDEHTVLGDAPGLYVRDLKAGIPV

SEQ ID NO: 29 - protein, 562 aa, Rhodococcus aetherivorans
MLDHVHKKLKSTLDPIGWGPAVKSVAGRAVRNPQAVTAATTEYAGRLVKIPAAATRVFNADDPKPPMPLDPRDRRFSDTAWRENPAYFSLLQSYLATRAYVEELTDAGAGDPLQDGKARQFANLMLDVLAPSNFLWNPGVLTRAFETGGASLLRGARYAVHDVLNRGGLPLKVDSDAFTVGENLAATPGKVVYRNDLIELIQYTPQTEQVHAVPILAAPPWINKYYILDLAPGRSLAEWAVQHGRTVFMLSYRNPDESMRHITMDDYYVNGIAAALDVVEEITGSPKIEVLSICLGGAMAAMAAARAFAVGDKRVTAFTMLNTLLDYSQVGELGLLTDPSTLDLVEFRMRQQGFLSGKEMAGSFDMIRAKDLVFNYWVSRWMKGEKPAAFDILAWNEDSTSMPAEMHSHYLRSLYGRNELAEGLYVLDGQPLNLHDITCDTYVVGAINDHIVPWTSSYQAVNLLGGDVRYVLTNGGHVAGAVNPPGKKVWFKAVGAPDAETGSPLPADPQVWDDAATRYEHSWWEDWTAWSNKRAGELVPPPAMGSAAHPPLEDAPGTYVFS

SEQ ID NO: 30 - protein, 561 aa, Rhodococcus aetherivorans
MMAQARTVIGESVEESIGGGEDVAPPRLGPAVGALADVFGHGRAVARHGVSFGRELAKIAVGRSTVAPAKGDRRFADSAWSANPAYRRLGQTYLAATEAVDGVVDEVGRAIGPRRTAEARFAADILTAALAPTNYLWTNPAALKEAFDTAGLSLARGTKHFVSDLIENRGMPSMVQRGAFTVGKDLAVTPGAVISRDEVAEVLQYTPTTETVRRRPVLVVPPPIGRYYFLDLRPGRSFVEYSVGRGLQTFLLSWRNPTAEQGDWDFDTYAGRVIRAIDEVREITGSDDVNLIGFCAGGIIATTVLNHLAAQGDTRVHSMAYAVTMLDFGDPALLGAFARPGLIRFAKGRSRRKGIISARDMGSAFTWMRPNDLVFNYVVNNYLMGRTPPAFDILAWNDDGTNLPGALHGQFLDIFRDNVLVEPGRLAVLGTPVDLKSITVPTFVSGAIADHLTAWRNCYRTTQLLGGETEFALSFSGHIASLVNPPGNPKAHYWTGGTPGPDPDAWLENAERQQGSWWQAWSDWVLARGGEETAAPDAPGSAQHPALDAAPGRYVRDLPAG

SEQ ID NO: 31 - protein, 566 aa, Gordonia spumicola
MTIAQNQAAAGEIAAPLDLLLVNSTKSFARRMTPSGPLARFGASLAKQPVVVAEKGAGLAKELGDIALGRSNRAPARGDKRFSDPAWTQNPLLRRIEQAYLAASDTAEQLYDAAELDWKDAEKVRFALDNLIEGLAPTNNILINPLGWKALIDTGGMSAYRGVNAFVRDMASKPRVPSMVDSDAFTVGETVATTRGSVVLRTRMFELIHYAPATTTVHEVPLLLVPPVINKFYIMDIAPKRSMIENFVANGQQVFAISWRNPKARHRDWGFDEYGQAIIDAIDATQVITGAETTNLSGTCSGGILAAMVLAHLAATGHGDKVGSLTLGVTVLDQSQAGFAASLTSERAAAAAIAQSSRVGYLDGRAMAEMFAWLRPTDLVWRYWVNNYIQGRTPPAFDVLFWNADTTRMAAALHKDMVMMGLGNDLVTAGQATMLGTPVDLGAVECDSYVIGGIADHICPWQATYRSAALLGGKDNRFVLSSSGHIASLVNPPGNPKASFRIAQVDHDADPDTWLATAEKRSDSWWNDHIEWLAERSGDRVNAPSALGAAGFEPLAPAPGTYVLES

SEQ ID NO: 32 - DNA, 1756 bp, synthetic construct
  source 1..1756: mol_type = other DNA
ggaaacaattgcacgtgcagagagacaatcaaatcatgagtaacaagaatagcgatgacttgaatcgtcaagcctcggaaaacaccttggggcttaaccctgtcatcggcctgcgtggaaaagatctgctgacttctgcccgaatggttttaacccaagccatcaaacaacccattcacagcgtcaagcacgtcgcgcattttggcatcgagctgaagaacgtgatgtttggcaaatcgaagctgcaaccggaaagcgatgaccgtcgtttcaacgaccccgcctggagtcagaacccactctacaaacgttatctacaaacctacctggcgtggcgcaaggaactccacgactggatcggcaacagcaaactgtccgaacaggacatcaatcgcgctcacttcgtgatcaccctgatgaccgaagccatggccccgaccaacagtgcggccaatccggcggcggtcaaacgcttcttcgaaaccggcggtaaaagcctgctcgacggcctcacacatctggccaaggacctggtaaacaacggcggcatgccgagccaggtggacatgggcgctttcgaagtcggcaagagtctggggacgactgaaggtgcagtggttttccgcaacgacgtcctcgaattgatccagtaccggccgaccaccgaacaggtgcatgagcgaccgctgctggtggtcccaccgcagatcaacaagttttatgtgtttgacctgagcccggataaaagcctggcgcgcttctgcctgagcaacaaccagcaaacctttatcgtcagctggcgcaacccgaccaaggcccagcgtgagtggggtctgtcgacttacatcgatgcgctcaaagaagccgtcgacgtagtttccgccatcaccggcagcaaagacatcaacatgctcggcgcctgctccggtggcattacctgcaccgcgctgctgggtcactacgccgctctcggcgagaagaaggtcaatgccctgacccttttggtcaccgtgctcgacaccaccctcgactcccaggttgcactgttcgtcgatgagaaaaccctggaagctgccaagcgtcactcgtatcaggccggcgtgctggaaggccgcgacatggccaaagtcttcgcctggatgcgccctaacgacctgatctggaactactgggtcaacaactacctgctgggtaacgagccaccggtcttcgacattcttttctggaacaacgacaccacccggttgcctgctgcgttccacggcgatctgatcgaaatgttcaaaaataacccactggtgcgcgccaatgcactcgaagtgagcggcacgccgatcgacctcaaacaggtcactgccgacatctactccctggccggcaccaacgatcacatcacgccctggaagtcttgctacaagtcggcgcaactgttcggtggcaaggtcgaattcgtgctgtccagcagtgggcatatcaagagcattctgaacccgccgggcaatccgaaatcacgttacatgaccagcaccgacatgccagccaccgccaacgagtggcaagaaaactcaaccaagcacaccgactcctggtggctgcactggcaggcctggcaggccgagcgctcgggcaaactgaaaaagtccccgaccagcctgggcaacaaggcctatccgtcaggagaagccgcgccgggcacgtatgtgcatgaacgttaacctgccggcctggttcaaccagtcggcagccgactagtgga

SEQ ID NO: 33 - DNA, 1756 bp, synthetic construct
  source 1..1756: mol_type = other DNA
ggaaacaattgcacgtgcagagagacaatcaaatcatgagtaacaagaatagcgatgacttgaatcgtcaagcctcggaaaacaccttggggcttaaccctgtcatcggcctgcgtggaaaagatctgctgacttctgcccgaatggttttaacccaagccatcaaacaacccattcacagcgtcaagcacgtcgcgcattttggcatcgagctgaagaacgtgatgtttggcaaatcgaagctgcaaccggaaagcgatgaccgtcgtttcaacgaccccgcctggagtcagaacccactctacaaacgttatctacaaacctacctggcgtggcgcaaggaactccacgactggatcggcaacagcaaactgtccgaacaggacatcaatcgcgctcacttcgtgatcaccctgatgaccgaagccatggccccgaccaacagtgcggccaatccggcggcggtcaaacgcttcttcgaaaccggcggtaaaagcctgctcgacggcctcacacatctggccaaggacctggtaaacaacggcggcatgccgagccaggtggacatgggcgctttcgaagtcggcaagagtctggggacgactgaaggtgcagtggttttccgcaacgacgtcctcgaattgatccagtaccggccgaccaccgaacaggtgcatgagcgaccgctgctggtggtcccaccgcagatcaacaagttttatgtgtttgacctgagcccggataaaagcctggcgcgcttctgcctgagcaacaaccagcaaacctttatcgtcagctggcgcaacccgaccaaggcccagcgtgagtggggtctgtcgacttacatcgatgcgctcaaagaagccgtcgacgtagtttccgccatcaccggcagcaaagacatcaacatgctcggcgcctgctccggtggcattacctgcaccgcgctgctgggtcactacgccgctctcggcgagaagaaggtcaatgccctgacccttttggtcaccgtgctcgacaccaccctcgactcccaggttgcactgttcgtcgatgagaaaaccctggaagctgccaagcgtcactcgtatcaggccggcgtgctggaaggccgcgacatggccaaagtcttcgcctggatgcgccctaacgacctgatctggaactactgggtcaacaactacctgctgggtaacgagccaccggtcttcgacattcttttctggaacaacgacaccacccggttgcctgctgcgttccacggcgatctgatcgaaatgttcaaaaataacccactggtgcgcgccaatgcactcgaagtgagcggcacgccgatcgacctcaaacaggtcactgccgacatctactccctggccggcaccaacgatcacatcacgccctggaagtcttgctacaagtcggcgcaactgttcggtggcaaggtcgaattcgtgctgtccagccgcgggcatatccgcagcattctgaacccgccgggcaatccgaaatcacgttacatgaccagcaccgacatgccagccaccgccaacgagtggcaagaaaactcaaccaagcacaccgactcctggtggctgcactggcaggcctggcaggccgagcgctcgggcaaactgaaaaagtccccgaccagcctgggcaacaaggcctatccgtcaggagaagccgcgccgggcacgtatgtgcatgaacgttaacctgccggcctggttcaaccagtcggcagccgactagtgga

SEQ ID NO: 34 - DNA, 1756 bp, synthetic construct
  source 1..1756: mol_type = other DNA
ggaaacaattgcacgtgcagagagacaatcaaatcatgtcgaacaagaactccgacgacctgaaccgccaggcgtcggagaataccctgggcctgaaccccgtgattggcctgcgcggcaaggacctcctgaccagcgcgcgcatggtcctgacccaggcaatcaagcaacccatccactccgtgaagcatgtcgcgcatttcggcatcgaactgaagaacgtcatgttcggcaagtccaagctgcagccggagagcgacgatcgccggttcaacgacccggcctggtcgcagaacccgctgtataagcgctacctccagacctacctggcctggcggaaggagctgcacgactggatcgggaactccaagctgtcggaacaggacattaatcgcgcccacttcgtcatcaccctgatgaccgacgcgatggcgccgaccaactcggccgcgaacccggcagccgtgaagcggttcttcgaaaccggcgggaagtccctgctggatggcctcacccatctggccaaggacctggtgaacaacggcgggatgcccagccaagtggatatgggcgcgttcgaggtgggcaagtccctgggcacgacggagggtgccgtggtgttccgcaacgatgtcctggaactgatccagtaccgtccgaccaccgagcaagtgcacgagcgtccgctcctggtcgtgccgccccagatcaacaagttctacgtgttcgacctgagccccgataagagcctggcccgcttctgcctctcgaacaaccaacagaccttcatcgtgagctggcgcaatcccaccaaggcgcagcgcgagtggggcctgtccacctacatcgacgccctgaaggaggccgtcgacgtggtgagcgccatcacgggcagcaaggacatcaatatgctgggcgcctgctcgggcggcatcacgtgcaccgcgctcctcggtcactacgccgccctgggcgagaagaaggtgaacgccctgacgctgctggtctgcgtgctggacaccaccctggacagccaggtggcgctgtttgtggacgaaaagaccctggaggcggccaagcgccacagctaccaggcgggtgtcctggagggccgcgacatggcgaaggtgttcgcctggatgcgcccgaacgacctgatctggaactactgggtcaacaactatctgctgggcaatgagccgcccgtgttcgatatcctgttctggaacaatgacacgacgcggctccccgcagcctttcacggcgatctgatcgaaatgttcaagaacaacccgctggtgcgcgccaacgcgctggaagtgtccggcacgccgatcgacctgaaacaggtcaccgccgacatctactcgctggccggcacgaacgaccacatcacgccgtggaagtcgtgctacaagtcggcccagctcttcggtggcaaggtcgagtttgtgctgtcgtcgcgcggccatatccagagcatcctgaatccgccgggcaacccgaaatcgcgctatatgacctcgaccgacatgccggccacggccaacgagtggcaggaaaactcgacgaagcacaccgactcgtggtggctgcactggcaggcctggcaggcggaacgcagcggcaagctgaagaagtcgccgacctcgctgggcaacaaagcctatccgtcgggcgaagcggcaccgggcacctacgtccacgaacgctgacctgccggcctggttcaaccagtcggcagccgactagtgga

SEQ ID NO: 35 - DNA, 1756 bp, synthetic construct
  source 1..1756: mol_type = other DNA
ggaaacaattgcacgtgcagagagacaatcaaatcatgagcaacaagaacaacgatgacttgcagaggcaagcgtcggagaataccctgggcctgaatccggtgatcgggctgcgccggaaggacctgctgacgagtgcgcgtatggtgctgggacaggcgattcgccaaccgctgcactccgccaagcatgtggcccactttggcctggaactcaagaacgtcatcttcggcaaatccggactccagccggagtcggacgaccgccgcttcaatgaccccgcatggagccaaaaccccctgtatcgccgctatctgcagacctacctggcctggcgcaaggagttgcacgactggatcgacaactcgaacctgtcggagcaggacatctcgcgtggccacttcgtgatcaacctcatgaccgaggcgatggcaccgacgaacaccgcagccaacccggcggccgttaagcgcttcttcgagacgggcggcaagtccttgctggatggcctgagcaacctggcgaaggacatggtcaacaatggcggcatgccctcccaggtcaacatggaggcgttcgaagtgggcaagaacctgggcaccagcgaaggcgctgtggtgtaccggaacgacgtcctggaactgatccagtacaagcccatcacggaacaggtccattcacgccccctgctggtggtcccaccgcagatcaacaagttctacgtgttcgacctgtccccggagaagtcccttgcccgcttttgcctccgctcgaacgtccagacgttcatcgtgtcgtggcggaacccgaccaagacacagagagaatggggcctctcgacctacatcgatgccctgaaggagacggtggacgtagtgctggcgatcacgggctccaaggacctgaacatgctgggtgcgtgctcgggcggcattacctgcactgcgctgctgggccattatgcggccctgggggagaacaaggtgaatgccctgaccctgcttgtctcggtcctggacaccaccctggatacgcaggtcgccctcttcgtcgatgaacagacccttgaaagcgcgaagcgccagagctaccaggccggtgtgctggaaggccgcgacatggccaaggtcttcgcctggatgcgcccgaacgacctgatctggaactactgggtgaacaactacctgctggggaatgaaccgccggtgttcgacatcctgttctggaacaacgacaccacgcgtctcccggcagcgtttcatggcgacctcatcgagctgttcaagagcaaccccttgacccgcgcggatgccctggaggtgtgcggcaccccgatcgacctgaagaaggttaccgccgacatctactctctggccggcacgaccgaccacatcacaccgtggcaagcgtgctaccgcagcgcacaactgttcggcggcaacatcgagttcgtgctgagcaattcgggccacatccagagcatactgaacccacctggcaacccgaaagcccgctacatgaccggctcggagctgccgacccaggccacggaatggcaggaaaacgcccacaagcacaccgacagctggtggctacactggcagaactggctcgccactcgctcgggtgagctcaagaaggcccccacgcgactgggcaatcgggcctatgccgcgggtgaagctgccccgggcacctacgtgcacgagcgctgacctgccggcctggttcaaccagtcggcagccgactagtgga

SEQ ID NO: 36 - DNA, 1756 bp, synthetic construct
  source 1..1756: mol_type = other DNA
ggaaacaattgcacgtgcagagagacaatcaaatcatgtcgaataagaacaatgacgagctgcagcgccaggcgtccgagaacaccctgggcctgaatccggtgatcgggatccgccggaaggatctgctgtcgtccgcccgcaccgtgctccgtcaagcggtgcgccagccgctgcattcggcgaagcacgtggcccatttcggcctggaactgaagaatgtgctgctgggcaagagctcgctggcgccggaaagcgacgaccgccgcttcaacgatccggcctggagcaacaacccgctgtaccgccgctatctgcagacctacctcgcgtggcgcaaggaactgcaggattggatcggcaacagcgatctgtcgccccaggacatctcgcgcggccagttcgtgatcaacctgatgacggaggcaatggccccgaccaacaccctgagcaatccggcagccgtgaagcggttcttcgaaaccggcggcaagtccctcctggacggcctgtcgaacctggcgaaagacctggtgaacaatggcggcatgcccagccaggtcaacatggacgccttcgaggtcgggaagaacctgggtacgtcggaaggcgcggtggtgtaccgcaacgacgtgctggagctgatccagtacaagcccatcaccgagcaagtgcatgcccgcccgctgctggtcgtgccgccgcagatcaacaagttctacgtgttcgacctctcgccggagaagagcctggcccgctactgcctgcgctcgcaacagcagaccttcatcatctcctggcgtaacccgaccaaggcccagcgcgagtggggcctctcgacctacatcgacgcactgaaggaggcggtcgacgcggtcctggcgattaccggctcgaaggacctgaacatgctcggcgcctgctcgggcggcatcacgtgcaccgccctggtgggccactatgccgccctgggcgagaacaaggtgaacgccctgaccctgctggtcagcgtcctggacacgacgatggacaaccaagtcgccctgttcgtggacgagcagacgctggaagccgccaagcggcactcgtaccaggccggtgtcctggaaggctcggaaatggcgaaggtgtttgcgtggatgcgccccaacgacctgatctggaactactgggtcaacaactacctcctgggcaatgagccgccggtgttcgacatcctgttctggaacaacgatacgacgcgcctgcccgccgcgtttcacggcgacctcatcgagatgttcaagtccaatccgctgacccgcccggacgccctggaagtgtgcggcaccccgattgacctcaagcaagtgaagtgcgacatctactccctggcgggcaccaacgaccacatcaccccgtggcagtcgtgctaccgctcggcccacctgttcggcgggaagatcgagtttgtcctgagcaactcgggccacatccagagcatcctcaacccgccgggtaacccgaaggcccggttcatgacgggcgccgatcgccccggcgatcccgtggcctggcaggaaaacgccaccaagcacgcggactcctggtggctgcactggcagagctggctgggtgagcgcgcaggggaactggagaaagcacccacgcgtctgggcaaccgcgcgtatgccgccggcgaagcgagcccgggcacctatgtccatgaacgctgacctgccggcctggttcaaccagtcggcagccgactagtgga

SEQ ID NO: 37 - DNA, 1756 bp, synthetic construct
  source 1..1756: mol_type = other DNA
ggaaacaattgcacgtgcagagagacaatcaaatcatgtcggacaagaacaacgaagatctgaagcgccaggccagcgaaaacaccctgggcctgaacccggtcatcggcattcgcggcaaggatctgctgacctcggcgcgcatggtgctggcacaagcgctgaagcagccgttccactcggccaagcacgtggcgcacttcggcctcgagctgaagaacgtgatgctgggccagtcggccctgaaaccggaggacggcgaccgtcgcttcgcggacccggcatggtcccagaatccgctgtaccggcgctatctgcagacctacctcgcctggcgcaaggagctgcatgactgggtggagcactcctccctcagcgagcaggatgcgtcccgcggcacgttcgtgatcaacctgatgaccgaggacatggccccgtcgaactccatggccaaccccgcggccgtgaagcgtttcttcgaaacgggcgggaagtcgctgctggacggcctgagccatctggccaaggacatggtgcacaacggcggtatgcccagccaggtgaacatggaagccttcgaagtgggcaagaatctggcgacgacggacggcgcggtcgtctttcgcaatgacgtgctggagctgatccagtataagccgatcacggaatcggtgcatgagcgcccgctcctggtcgtgccgccgcagatcaacaagttctacgtgttcgacctgtccccggacaagtcgctggcacgctttctgctgcgctcccaggtccagacgttcgtcgtcagctggcgcaaccccaccaaggcccaacgcgagtggggcctgtcgacctacatcgaagccctgaaggaggcgatcgacgtgatttgcgcgatcaccggctcgaaggacgtcaacatgctcggtgcctgctcgggtgggctgaccaccgcctcgctcctgggccattacgccgcgctcggccaacccaaggtcaatgccctgaccctgctggtgtcggtcctggatacgcagctggatacccaggtcgccctgttcgcggacgaaaagacgctcgaacggggccaacgccgcagctatcaggcgggcgtcctggagggcagcgacatggccaaggtgtttgcctggatgcggcccaacgatctgatctggaactactgggtgaacaactacctcctcgggaacgagccgccggtgttcgacatcctgtactggaacaacgacaccacccggctgcccgcagccctgcatggtgagttcatcgagatgttccagaccaatccgctgacccgtccgggcgcactggaagtctgcggcaccccgatcgatctgaaacaggtgacgtgcgacttcttcgtggtggcgggcaccaccgaccacatcaccccgtgggacagctgctacaagtcggcccacctgttcggcggcaagtgcgagttcgtgctgtcgaacagcggccacatccagagcatcctgaatccgcccggcaacccgaaagcccgctacatgaccaactcggagatgccgctggaccccaaggcgtggcaggaatcgagcacgaagcacgcggacagctggtggctgcactggcagtcgtggctggcggaacgctcgggcgaaaccaagaacgccccgcgcgccctgggcaacaagaagttcccggccggcgaagccgccccggggacgtatgtgcacgagcgctgacctgccggcctggttcaaccagtcggcagccgactagtgga

SEQ ID NO: 38 - DNA, 1774 bp, synthetic construct
  source 1..1774: mol_type = other DNA
ggaaacaattgcacgtgcagagagacaatcaaatcatgaccaagacggcggaaccgaaaatcgccctggtgatccccgatgccaccccggaggaagaggaccgtgccggtggcttcggtgcgcggaatgcactgaacgccgtgaccggtgtcgtcgggcaagggcgcgtggtcctggaggaatccctgcgtctgggccgcgaactcacgaagatcaccgtcggccgcagcgatgtcggtccggcagcaggcgatcggcgtttcacggaccaagcctggacgaacaatccgatctatcgccgtgtgcagcagacctatctggcgtcggtcgacgccgtggagagcgtcgtggaagacctgggccggcgtgtcgacgatcgtcacgcgcgggaagccgcctttgtgtcgaccgtgctcacgtcggccctcgcccccacgaactatctccccaccaaccccgccgccgtgaaagaagcattcgataccggcggcatgagcctcgtccgtggggcgcgcaactatgtcagcgatctgcgccataatggcggcatgccgcggatggtcgacccggatgcgttcaccgtgggcgtggatctggcggtcacgccgggtgccgtcgtgtcgcgtgacgaagtcgccgaggtcctccagtacacgcccaccaccgaaaccgtgtatgagcgcccggtgctggtggtgcccccgccgattggccgttactatttcctggacctgcggccgggtcgctcctttgtggaacacgccgtctcccgcggtctgcaaacctttatgctcgcgtggcgtaatccgcaggcggaacagtcggactgggatctggacacctatgcccagcgcgtgagcgacgccatcgatgaagtgcgcgagattaccggctcggacgatgtgaacgtgattggtttttgcgccggcggcctcattaccacggcgctgctgaatcatctggcggccacgggtgacacccgtgtgcacagcgtgagctatgcagtgaccatgctcgacttcgccgacccggccggcctggcagcattttcgggcccgcgtctgctgcaactggtgaagggccgctcccgccgcaacggtattatcagcgcccgcgatatgggttcggcctttacctggatgcgtcccaacgatctggtgttcaactatgtcgtgaataactacctgatgggccgcacgccgccggcattcgatatcctctcgtggaacgcggacggtaccaacctccccggtgcgctgcacgtgcaatttctggacatcttcgagaataacaccctggcgacccccggggcaatgaccgcactcggtacgcccgtcgacctgggtcgcatcacggtcccgaccttcgtgtccggggcgatcgcagatcatctgacgagctggaagaactgctaccgtaccacgcaactgctgtcgggtgacacgaagtttgtgctctccttctcgggccacatcgcctccctcgtcaatccgccgggtaatccgaaatcgcattattgggaaggcggcgaacccggtcccgacccggaagcctggctggatgcggcaacgaagaaaacgggttcgtggtgggagtcctgggcggactgggtgagcgagcgtgcaggcgagcgcatcgtcgcaagcacgcgtctgggctcggacgagcataccgtgctgggtgacgcacccggtctgtatgtccgtgacctgaaagcgggtatcccggtctgacctgccggcctggttcaaccagtcggcagccgactagtgga

SEQ ID NO: 39 - DNA, 1765 bp, synthetic construct
  source 1..1765: mol_type = other DNA
ggaaacaattgcacgtgcagagagacaatcaaatcatgttggatcacgtgcataagaagctcaagtcgaccctggatcccatcggctggggaccggccgtaaagtcggtggcaggccgcgctgtgcgcaacccgcaagccgtgaccgccgccaccaccgaatatgcgggccgcctggtgaagatcccggccgccgcgactcgcgtcttcaacgctgacgacccgaagccgccgatgcccctggacccgagggaccgccggttcagcgacaccgcctggcgcgaaaacccggcctacttctcgctgctgcagtcgtacctggccacccgcgcctacgtggaagaactgaccgacgcgggcgccggtgaccccctgcaggacggcaaagcccgtcagtttgcgaacttgatgctggacgtcctggccccctccaacttcctgtggaacccgggcgttctgacccgcgcgttcgaaacgggcggggcgagccttcttcgaggcgcccgctacgccgtgcatgacgtgctgaatcgcggcgggctgccgctgaaggtggactcggacgcgtttacggtgggggagaacctggccgcgacgcccggcaaggtggtgtaccgcaacgacctgatcgagctcatccagtataccccgcaaacagagcaggtccacgccgtcccgattctggccgccccgccgtggatcaacaagtattacatcctggacctagcgccgggccgcagcttggcggaatgggcggtgcagcacggcagaaccgtcttcatgctgagctaccgcaatccggacgagtcaatgcgccacatcaccatggacgactactacgtcaacggcattgcggcggccctggacgtggtggaggagatcaccggctccccgaagatcgaagtgctctccatctgcctgggcggagcgatggccgcgatggcagcggcgcgtgcgttcgcggtcggcgacaaacgcgtgacggctttcaccatgctcaacacgctgctggattatagccaggtcggcgagctgggcctgctgactgaccccagcaccctggacctcgtcgagttccgtatgcgccagcagggcttcctgagcggcaaggagatggccggcagcttcgacatgatccgcgccaaggatctggtcttcaactactgggtcagccggtggatgaagggcgagaagccggcagcgttcgacatcctcgcctggaacgaggactccacgtcgatgcctgccgagatgcactctcactacctccgctcgctgtacggtcggaacgagctggcggagggcctgtacgtcctcgatggccagcccctgaacctgcacgacatcacctgcgacacgtacgtcgtcggcgccatcaacgaccacatcgtgccgtggacgtcgtcgtaccaggccgtgaacctgctggggggcgatgtgcggtatgtcctcacgaatggcggccatgttgccggtgcggtgaacccgccgggcaagaaggtctggttcaaggccgtgggtgccccagacgccgagacgggctcgcccttgccagcagatccccaagtgtgggacgatgcagcgacccgctatgaacactcctggtgggaagattggaccgcctggtccaataagcgcgccggcgaactggtgccccctccggcaatgggcagtgcagcccatccgccactggaagacgcgccgggcacctacgtgttctcgtgacctgccggcctggttcaaccagtcggcagccgactagtgga

SEQ ID NO: 40 - DNA, 1762 bp, synthetic construct
  source 1..1762: mol_type = other DNA
ggaaacaattgcacgtgcagagagacaatcaaatcatgatggcccaagcgcgcaccgtaatcggcgaatcggtggaggagtccattgggggcggcgaggacgtcgctccgccgcgcctgggcccggcggttggcgcccttgcagacgtgtttggccatggtcgggcggtggcacgtcacggcgtcagcttcggccgcgaactggcgaagatcgccgtgggccgctcgacggtggccccggccaaaggcgaccgcaggttcgccgacagcgcgtggtcagcaaatcccgcctatcgccggctcggccaaacctacctggcagccacggaggcggtggatggcgtggtggatgaggtgggccgcgcaatcggaccgcggcgaacggcggaggcgcgcttcgccgccgacatattgaccgctgcgctggccccgacgaattacttgtggaccaatcccgcggccctgaaggaggccttcgacacggccggtctgtctctcgcccgtgggaccaagcacttcgtgtcggacctgatcgagaaccgcggcatgccctcgatggtccagcggggcgccttcacggtcggcaaggatctggcggtgactcccggcgccgtcatctcgcgcgacgaggtcgcggaagtgctgcagtacaccccgaccaccgagactgtccgccgtcgccccgtgctggtcgtgccgccccctatcggccgctactacttcttggacctgcggcccggccgctcgttcgtcgagtacagcgtgggcagaggcctgcagacgttcctgctgagctggaggaacccgaccgccgaacagggcgactgggacttcgacacctatgccggccgcgtcatccgcgccatcgacgaagtgcgcgaaatcaccggcagcgatgacgtgaacctgatcgggttctgcgccggcggcatcatcgccaccacagtgctgaaccacctggcggcccagggcgacacccgggtccactcgatggcctatgccgtcaccatgctggactttggcgatccggccctgctgggcgcgtttgcccgcccgggcctgattcgcttcgccaagggccgctcccgccgtaagggcatcatcagcgcccgcgacatgggctccgcgttcacatggatgcgcccgaacgacctggtcttcaactacgtcgtgaacaactacctgatgggccgcacccctccggcgttcgacatcctcgcgtggaacgatgacggcacgaacctgccgggagccctgcacggccagttcctggacatcttccgggacaacgttctcgtggaaccgggtcgcctagcggtgctggggaccccggtggacctgaagtcgatcaccgtccccacgttcgtctccggggcgatcgcggaccacctgacggcctggcgcaactgctatcgcaccacgcagctgctcggcggtgaaacggagttcgcgctgagcttctccggccatatcgccagcctcgtgaacccaccgggcaatccgaaggcccactactggaccggcggcaccccgggtcccgacccggatgcgtggctggagaacgccgaacgccagcaaggctcgtggtggcaggcctggtcggactgggtgcttgcgcgcggtggcgaagaaaccgcagctccggatgcgccggggagtgcccagcatcccgccctcgacgcagctccaggccgatacgtgcgcgacctgccggcgggctgacctgccggcctggttcaaccagtcggcagccgactagtgga

SEQ ID NO: 41 - DNA, 1777 bp, synthetic construct
  source 1..1777: mol_type = other DNA
ggaaacaattgcacgtgcagagagacaatcaaatcatgaccatcgcccagaaccaagccgccgcgggcgaaatcgccgccccgctggaccttctgctggtgaacagcaccaagagcttcgcccggcgtatgaccccgtcgggcccgctggcacgttttggcgcatccctggcgaagcaacccgtggtcgtggcggagaagggcgcgggactggccaaggaactgggcgacatcgccttgggccgcagcaatcgcgcgcctgcacgcggcgacaagcgcttcagcgatcccgcgtggacgcagaacccgctcctgcgccgcatcgaacaggcctatctggccgcgtcggacaccgcggagcagctgtacgacgccgcggagctcgactggaaggacgccgaaaaagtgcgcttcgccctggacaacctcatcgagggcctcgcccccaccaacaacatcctgatcaacccgctgggctggaaggccctgattgacacgggcggcatgtcggcttaccgcggggtcaacgcgttcgttcgcgacatggcctcgaagccccgcgtcccgtcgatggtcgacagcgacgccttcaccgtgggcgaaaccgtggcaaccacgcgcggctcggtggtcttgaggacccggatgttcgagctgatccactatgcccccgcgaccaccacggtgcacgaggtccctctgctgctggtaccgccggtgatcaacaagttctacatcatggacatcgcgccgaagcggagcatgatcgagaacttcgtggcgaacggccagcaggtgttcgcgatctcgtggcgcaatcccaaggctcggcaccgcgattggggctttgacgagtacggccaggccatcatcgacgcgatcgacgccacgcaggtgattaccggcgccgaaaccaccaacctgtccggcacctgctccggtggcatcctggcagcgatggtcctggcccaccttgccgccactggccatggcgacaaggtcggcagcctgacactgggcgtcaccgtgctggatcagtcgcaggccggctttgcggcgtctctgacgtccgaacgcgccgcggctgcagcgattgctcagagctcccgcgttggctacctggatgggcgagccatggcggagatgttcgcctggctgcgcccgacagatctcgtgtggcgctactgggtgaacaactacatccagggacgcacgcccccggccttcgacgtcctgttctggaatgccgatactacgcgcatggccgccgcgctgcacaaggacatggtcatgatgggcctggggaacgacctggtcacggccggtcaggcgaccatgctgggtacgccggtggatctgggggcggtggagtgcgactcatacgtgatcggcggcatcgcggaccacatatgcccctggcaggccacctaccgttcggcggccctgctcggcggcaaagacaaccgcttcgtcctatccagctcgggccatatcgcctcgctcgtgaacccgccgggcaatccgaaggcctccttccgcatcgcgcaagtggaccatgacgccgacccggacacctggctcgccacggcggaaaagcggagcgattcgtggtggaatgaccacatcgagtggctggccgaacgcagcggcgacagagtgaacgcgccaagtgccctgggtgccgcaggtttcgagccgttggccccggcaccaggcacctatgtgctggaatcgtgacctgccggcctggttcaaccagtcggcagccgactagtgga

SEQ ID NO: 42 - DNA, 1765 bp, synthetic construct
  source 1..1765: mol_type = other DNA
ggaaacaattgcacgtgcagagagacaatcaaatcatgaccacgaccgccaaagtggatgaactcgccgcacccctcgatctgctcctgacgtcggcgacgaaaccgtttgcatcgcgtatgatgcccaatgcaacgtgggcacggtttgcgggtaatctggcacaacatccgggtgccgtcgcggatcgcgtcggggcactcacgcgggaactcggtaatattgcggtcggtaaatcccatcgtgcccccggtcgggcggataaacgcttttccgatccggcctggcaagaaaatcccctgctgcatcgtattatgcaagcgtatctcgcaggtagcgaaacggccgaagaactgctggcagatgcacagctggactggcgggataaagaaaagatgcaatttgtcattgataatttcgtggaagggctcgcaccctcgaataatcccctcattagccccctgggttggaaagccctcattgatacgggtggtctctcggccgtgcgtggtgcacgcgcatttgcacgtgatatgctgtccaaaccgcgtgtcccggccatgattgaaccggatgcgtatgccgtcggtgaagatctggcagtgacgaaaggcgcagtggtgctccaaacgagcgtctttgagctgattcaatatgcgccccaaacgccgaaagtccgtgccattcccctgctgatggtcccgcccgtcattaataaatattatgtgatggatattgcaccgggccgttcgatgattgaatattttgtgcaacaagggcaacaagtgtttacgatttcctggcgcaatccccaagcacggcatcgtgactggggttttgatacgtacggtgccgccattgtcgaagccatggatgcggccgagaaaattacgggtacggattcgacccatctcctggcgacgtgctccggtgggattctcgccgccatgaccgccgcgcatctggcggaaattggggaaggtgatcgtgtggccggtctgaatctcgccgtgacggtcctcgatgaaacccgggcgggttttgccgcggcagcaatgtcggatcgggcagcccaagccgcaattcgggtgagctcccgcaaagggtttctcgatggtcgtgatatggccgaaatgtttgcgtggctgcgtcccacggatctcgtctggcgttatgtcgtcaataattatgtgcaaggtcgtaaaccggcagcctttgatgtcctgttttggaatgcggatacgacgcgtatggcagcagcactgcatcgggatctcgtcctcatgggcctgcgtaatgcactggtgaccccgggtggtgtgtcgatgctcggttcgcccgtcgatctggggaaaattacggccgatgcgtatattgtgggtggtattgcagatcatatttcgccctggcaagcgacgtatcggagcgcccggctcctcggttcgaaagataatcgttatgtcctgagcacgaatggtcatattgccgccctggtcaatcccccgggcaatccgaaagcaagctttcggaccggttccgtggatgcggaagacgcacaacaatggctcgattccgcagagaaacatgcggattcgtggtggcccgattataccgcgtggctcgcagaacgttcgggcgcagaagtggatgcaccgaaagcactgggcggcgaagatctgcccccgctcggtccggcgcccggttcgtatgtcatggagaaataacctgccggcctggttcaaccagtcggcagccgactagtgga

SEQ ID NO: 43 - DNA, 1777 bp, synthetic construct
  source 1..1777: mol_type = other DNA
ggaaacaattgcacgtgcagagagacaatcaaatcatgcgtccggaaatcacggatcgctcgggtcaagtccagaacgtcggcctggaccaactcctgaccgaagcggccagcgcggagtcgcgttttgtgccgggtgccgagttcctgaaggccgccggtggtctggcactgcgtccccggctgctcgccaatcaaaccgcgaccgtggcagccgatctggcgcgggtgattgccggtcgttccggccgtacgcccccgaaaggtgactcccgttttcgcgatccggcatggacgcaatcgtggctgtttcgccgtatttgccagggttacctctccatcagcgattatgcgcgtgcgctggccgacgaaagcggcctcgattgggcagatcacgaacgcctgcgcctggtcgtggacaatctgattgacgcgctggccccgaccaactttcccctcacgaaccccacggtctggaagacgaccattgaccggggcggtgagaattttgtcaccggtgcacgtgccgcggtccgcgatgcccgctcgcccatcaaactgcccgcgagcgtcgaccgcaccccgttcgaggtgggcaaaaccatggccgccagcccgggcgcagtggtgcgtcgcgatgaccgctttgaactgatccaatacgagccgcgtgccgaagaggtccacaaggtccccgtgctcctgattccgcccatgatctcgaagttttatgtggtggacctctcgcccggtaagagcatggtcgagttcctgggtgaccggggtctgcaaccgttcgccctgtcgtgggcgaatccgacgcgtgacaacgcaggttggaacctccaagattatctggagtccattgtcgaagccattgagacgacccgtgaaattgccggcgccgacgccgtgcatgtggtggcattttgcgccggtggcattgcgacgaccacggcggtcgcgcatctggcagcgctgggccacattgatcgtgtggcctcgctctccctgatggtgaccgtgctggatgtgcggcgtgggggtccgattctgagcatcgcctcgccggatgtcgcgaaggccgcgaaggcgaagatcaagcgcaagggctacctggccggcaccgagctgtcgcgtaccttcgcatggctccgcccgaacgacatggtctggaacaacttcgtcaataactactacctgggtaataagcccccggcgctggatctgctcttctggaacctcgactcgatgaatatgccggcaggcctgcacgcggatctggtggacctggccctggcaaacccgctcgccaatccgggggcgctgcgtgtgctgggcaccccgattgacctggcccagatcacgtgcgatgcctacatcgccgcaggggagaccgatcacctgacgccgtggccgtcgtgctatcgcagcgtcgagatgctcggtggcaagacgcggttcgcgctcagcacctcggggcatatcgcagcggtgatccatcccccgggtaacccgaagagcgcgtaccgtattggcgacgaatcctgcccgacccccgaagaatggctccgctccgcgcaagtgcacaaaggcacctggtggcaggactgggcaccctggctggcggaacgtgccggcgaaaagaccacggcccccgaccgtctgggcaattcccgttacacgcccctggacccggccccgggtacctatgtgtttaaacaaagccagggttgacctgccggcctggttcaaccagtcggcagccgactagtgga

SEQ ID NO: 44 - DNA, 1717 bp, synthetic construct
  source 1..1717: mol_type = other DNA
ggaaacaattgcacgtgcagagagacaatcaaatcatgctgctgattcgcagcgccactggcttcggccgccgaatggtgccgaacggcgcctgggtccgaacggcaggcaacctgatcaagcgtcctgggaccgtcgccagccgcgtcggagccctggtaggggaactgacggacattgcgttgggcgcctcggacagagccccgggacgcgccgataagcgctttgcggacccggcctggtcccagaacccggtgctgcaacgggtcatgcagacctatctggccaccagtgagacggcccagcacctgctggatgacgccgagctggactggagggaccgcgaacagatgcagttcgtgatcgacaacgtggtggaaggcggctcgccgtccaacaacatcctgctgtcgccgcttggctggaaggcgatgatcgatactggcggtctgtcggccgtccgtggcgcgcggaacttcgtgcgtgatatgcgctcggcaccacgcgtgccggcaatggtggacgcgaacgccttcgccgtgggcgattcgctggccgttacccccggctccgtggtgctgaagacgcgcgtgttcgagctgatccagtacgctccggcgaccccgaccgtcaccaccgtgcccctgctcgtgataccgccggtcatcaacaagtactacgtcctcgatctggccccccatcgcagcctcatggagtacctggtgtcgcagggcatccagccgttcgtgctctcatggcgcaatccgcacaagcgtcatcgcgactggggcttcgacacctatggcggctccatgatcgaggccatggacgcgatcggcgacatcaccggctcggaccgcgtgcacctgctagggacctgcagcggcggcatgctggcgtcgatggtcgccgcgcatttgacggcaatcggccagggtgaacgcctggcgtcgttggcgcttgcggtgacggtgctggaccagagcaaggccggtttcgccgcggcagcgctggacgagaagagcggccaagcagccatccgcaagtcggcccggaagggctacctcgacggtgcggctctggctgaggtcttcgcctggctccgcccgaccgatctggtctggcgctactgggtcaacaactacatccagggccgcgacccggcggccttcgacgtcctctactggaacgcggacacgacccgcatgaccgccgccctgcaccgcgacatggtgacgacgggcatgacgaacgccctggcccatccgggcgcagctaccatgctggggacagaggtggacctgtcgaaggtgaccgccgacatctacgtggtcggcggcgtgaccgaccacatctgcccgtggcccgccacctatcggtcctcccgcctgttcggcagcgacgacgtgcgctatgtcctctcgagctctggccacatcgccgcgatcgtcaatcccccaggcaatccccgggcgagcttccgctttggcccgccggactcggaatcacacgaagagtgggccgaaagcgcggaaaaggcggcggactcgtggtggccggattacgccgcctggctgaagcaacgcggcgaggacaaggacgcgcccgactccctgggcagcaaagcgttccccgttcgcagccctgcccccggtgaatacgtgcacgagcactgacctgccggcctggttcaaccagtcggcagccgactagtgga

SEQ ID NO: 45 - DNA, 1795 bp, synthetic construct
  source 1..1795: mol_type = other DNA
ggaaacaattgcacgtgcagagagacaatcaaatcatgacgaccacggaagaagaagcagcggccgcggcagaagggagcagcctcgcggaagaactgagcacgcccctggatctcctgctggcggatgcggggcggtcgcccattcgtcggtttctcccgggtatgagcggtgtccgctttgcggcaggtctcgcgcgtcggccgcataaagtggtggggcggacggcgggtctgggtgtggaactcgccaaagtgggtctgggtcgttcggaactggcgcccgcacccaaagatcggcgttgggcggatgaagcatgggcgaagaatcccctctttcgccgcaccctgcaaggttatctcgcgtggggtcaagcggtccgtggcctcgtggatgatgcggatctggattggggcgatggccatcgtattgggtttctcgcggataatctcgtggaagccatggcgcccacgaataatccggccctgaatccgaaagtgctgaaacgtacgctggatacgggtggtggtaatctcctcgaaggtggtaaacgtctggtccgggattttgcgacggcaccccgtgtccccagcatggtggaagcggatgcgtttgaagtgggtaaagatattgccgtgacgccgggcgcagtggtgctccgtacggatgtgtttgaactgattcaatattcgccccaaaccccgcaagtccgggaagtgcccctgctgattgtgccgcccaccattaataaatattatgtggtcgatctggcggccgaacgttccatgattgaacatctggtccggtcgggtctgcaagtgtattgcatttcgtggcgtaatccggatgcgcgccatgcagcatgggatctggatacgtatggtcaagcggtgctcgatgcgctggatggtattgaacaaatttcgcggcaagataaaacggcgctcctggggatttgcagcggtggcatgattgcgtccatggtcatggggcatctggccgcgacgggtaaactggatcgtgtggcggcattttcgctcatggtgaccgtgctcgatcaagaacgggcgggtgtgacgtcggcactcctcagccataaagcagcagcagcatcgacccgtgcgagcgcggaaaaaggttatctggatggtcgcgtcctcgcagaagtgtttgcatggctccgtccgaatgatctcatttggaattattgggtgaataattatctcatgggtcatgcacccaaagcctttgatattctcttttggaatgcggatcccgtgcgtatgtccgccggtatgcatcgtgattttatggatctcgcgtttcgtaatgcactcgtggaacccaatgcagcgaccatgctggataccccggtcgatctgggtaaagtgacgacggattcgtatgtggtcgcagggattgcagatcatctgtgccaatgggaaagctgctatgcatcgacgcaactcctcggtggtacgtcgaaatttgtcctcagcacgtcggggcatattgcagcgatggtgaatccgcccgggaatcccaaagcgaattttcgtacggcggaacaaaatcccccggaagcccaagattggctcgcgggtgcccatcaagtcccggggagctggtgggatgattatgcaggttggctcgcagaacgctgcggtgatgaacgtggtaaaccgcgtcgtctcggttcggcacaacatgaaccgctgtgcgaagcgcccggtacgtatgtgcatgatcgttaacctgccggcctggttcaaccagtcggcagccgactagtgga